European Patent Application EP 4 483 874 A1, published January 1, 2025. Title: Novel compound and composition for preventing, alleviating or treating bacterial inflammation and inflammasome-mediated disease comprising the same as an active ingredient. Applicant: Quorum Bio Co., Ltd. The sequence listing filed with the application follows.

SEQUENCE LISTING (16 sequences)

SEQ ID NO: 1 - DNA, 18 bp, synthetic construct
  misc_feature 1..18: note = synthetic_primer_Lysine-gingipain (Kgp)_forward
  source 1..18: mol_type = other DNA
caaccaaagccaagaaga

SEQ ID NO: 2 - DNA, 18 bp, synthetic construct
  misc_feature 1..18: note = synthetic_primer_Lysine-gingipain (Kgp)_reverse
  source 1..18: mol_type = other DNA
cgaagctgaagtaggaac

SEQ ID NO: 3 - DNA, 20 bp, synthetic construct
  misc_feature 1..20: note = synthetic_primer_Arginine-gingipain A (RgpA)_forward
  source 1..20: mol_type = other DNA
gctctttccataaacgtaag

SEQ ID NO: 4 - DNA, 18 bp, synthetic construct
  misc_feature 1..18: note = synthetic_primer_Arginine-gingipain A (RgpA)_reverse
  source 1..18: mol_type = other DNA
gacactcgtgagatgaag

SEQ ID NO: 5 - DNA, 21 bp, synthetic construct
  misc_feature 1..21: note = synthetic_primer_Arginine-gingipain B (RgpB)_forward
  source 1..21: mol_type = other DNA
cttccactttcacatccttta

SEQ ID NO: 6 - DNA, 18 bp, synthetic construct
  misc_feature 1..18: note = synthetic_primer_Arginine-gingipain B (RgpB)_reverse
  source 1..18: mol_type = other DNA
ctgacgatggtgatatgg

SEQ ID NO: 7 - DNA, 19 bp, synthetic construct
  misc_feature 1..19: note = synthetic_preimer_16s rRNA_forward
  source 1..19: mol_type = other DNA
acgagtattgcattgaatg

SEQ ID NO: 8 - DNA, 21 bp, synthetic construct
  misc_feature 1..21: note = synthetic_premer_16s rRNA_reverse
  source 1..21: mol_type = other DNA
accctttaaacccaataaatc

SEQ ID NO: 9 - DNA, 20 bp, synthetic construct
  misc_feature 1..20: note = synthetic_primer_TNF-a_forward
  source 1..20: mol_type = other DNA
cagagggaagagttccccag

SEQ ID NO: 10 - DNA, 22 bp, synthetic construct
  misc_feature 1..22: note = synthetic_primer_TNF-a_reverse
  source 1..22: mol_type = other DNA
cctcagcttgagggtttgctac

SEQ ID NO: 11 - DNA, 19 bp, synthetic construct
  misc_feature 1..19: note = synthetic_primer_IL-6_forward
  source 1..19: mol_type = other DNA
gtgaggaacaagccagagc

SEQ ID NO: 12 - DNA, 18 bp, synthetic construct
  misc_feature 1..18: note = synthetic_primer_IL-6_reverse
  source 1..18: mol_type = other DNA
tacatttgccgaagagcc

SEQ ID NO: 13 - DNA, 22 bp, synthetic construct
  misc_feature 1..22: note = synthetic_primer_IL-8_forward
  source 1..22: mol_type = other DNA
ttttgccaaggagtgctaaaga

SEQ ID NO: 14 - DNA, 21 bp, synthetic construct
  misc_feature 1..21: note = synthetic_primer_IL-8_reverse
  source 1..21: mol_type = other DNA
aaccctctgcacccagttttc

SEQ ID NO: 15 - DNA, 19 bp, synthetic construct
  misc_feature 1..19: note = synthetic_primer_GAPDH_forward
  source 1..19: mol_type = other DNA
gaaggtgaaggtcggagtc

SEQ ID NO: 16 - DNA, 18 bp, synthetic construct
  misc_feature 1..18: note = synthetic_primer_GAPDH_reverse
  source 1..18: mol_type = other DNA
agatggtgatgggatttc